European Patent Specification EP 3 972 643 B1, published May 14, 2025. Title: METHODS OF TREATING PARAPROTEINEMIC NEUROPATHY. Applicant: ARGENX BVBA. The sequence listing filed with the application follows.

SEQUENCE LISTING (31 sequences)

SEQ ID NO: 1 - protein, 752 aa, homo sapiens
MGPLMVLFCLLFLYPGLADSAPSCPQNVNISGGTFTLSHGWAPGSLLTYSCPQGLYPSPASRLCKSSGQWQTPGATRSLSKAVCKPVRCPAPVSFENGIYTPRLGSYPVGGNVSFECEDGFILRGSPVRQCRPNGMWDGETAVCDNGAGHCPNPGISLGAVRTGFRFGHGDKVRYRCSSNLVLTGSSERECQGNGVWSGTEPICRQPYSYDFPEDVAPALGTSFSHMLGATNPTQKTKESLGRKIQIQRSGHLNLYLLLDCSQSVSENDFLIFKESASLMVDRIFSFEINVSVAIITFASEPKVLMSVLNDNSRDMTEVISSLENANYKDHENGTGTNTYAALNSVYLMMNNQMRLLGMETMAWQEIRHAIILLTDGKSNMGGSPKTAVDHIREILNINQKRNDYLDIYAIGVGKLDVDWRELNELGSKKDGERHAFILQDTKALHQVFEHMLDVSKLTDTICGVGNMSANASDQERTPWHVTIKPKSQETCRGALISDQWVLTAAHCFRDGNDHSLWRVNVGDPKSQWGKEFLIEKAVISPGFDVFAKKNQGILEFYGDDIALLKLAQKVKMSTHARPICLPCTMEANLALRRPQGSTCRDHENELLNKQSVPAHFVALNGSKLNINLKMGVEWTSCAEVVSQEKTMFPNLTDVREVVTDQFLCSGTQEDESPCKGESGGAVFLERRFRFFQVGLVSWGLYNPCLGSADKNSRKRAPRSKVPPPRDFHINLFRMQPWLRQHLGDVLNFLPL

SEQ ID NO: 2 - protein, 9 aa, artificial
  Artificial
EDDHDAFAY

SEQ ID NO: 3 - protein, 17 aa, artificial
  Artificial
DINPNYESTGYNQKFKG

SEQ ID NO: 4 - protein, 5 aa, artificial
  Artificial
DYNMD

SEQ ID NO: 5 - protein, 9 aa, artificial
  Artificial
QHSRELPYT

SEQ ID NO: 6 - protein, 7 aa, artificial
  Artificial
LASNLKS

SEQ ID NO: 7 - protein, 15 aa, artificial
  Artificial
RASKSVRTSGYNYMH

SEQ ID NO: 8 - protein, 118 aa, artificial
  Artificial
EVQLVQSGAEVKKPGASVKVSCKASGYTFTDYNMDWVRQATGQGLEWIGDINPNYESTGYNQKFKGRATMTVDKSISTAYMELSSLRSEDTAVYYCAREDDHDAFAYWGQGTLVTVSS

SEQ ID NO: 9 - protein, 111 aa, artificial
  Artificial
DNVLTQSPDSLAVSLGERATISCRASKSVRTSGYNYMHWYQQKPGQPPKLLIYLASNLKSGVPDRFSGSGSGTDFTLTISSLQAEDAATYYCQHSRELPYTFGQGTKLEIK

SEQ ID NO: 10 - protein, 330 aa, homo sapiens [sequence omitted]

SEQ ID NO: 11 - protein, 329 aa, homo sapiens
ASTKGPSVFPLAPSSKSTSGGTAALGCLVKDYFPEPVTVSWNSGALTSGVHTFPAVLQSSGLYSLSSVVTVPSSSLGTQTYICNVNHKPSNTKVDKKVEPKSCDKTHTCPPCPAPEAAGGPSVFLFPPKPKDTLMISRTPEVTCVVVDVSHEDPEVKFNWYVDGVEVHNAKTKPREEQYNSTYRVVSVLTVLHQDWLNGKEYKCKVSNKALPAPIEKTISKAKGQPREPQVYTLPPSRDELTKNQVSLTCLVKGFYPSDIAVEWESNGQPENNYKTTPPVLDSDGSFFLYSKLTVDKSRWQQGNVFSCSVMHEALKFHYTQKSLSLSPG

SEQ ID NO: 12 - protein, 327 aa, homo sapiens
ASTKGPSVFPLAPCSRSTSESTAALGCLVKDYFPEPVTVSWNSGALTSGVHTFPAVLQSSGLYSLSSVVTVPSSSLGTKTYTCNVDHKPSNTKVDKRVESKYGPPCPSCPAPEFLGGPSVFLFPPKPKDTLMISRTPEVTCVVVDVSQEDPEVQFNWYVDGVEVHNAKTKPREEQFNSTYRVVSVLTVLHQDWLNGKEYKCKVSNKGLPSSIEKTISKAKGQPREPQVYTLPPSQEEMTKNQVSLTCLVKGFYPSDIAVEWESNGQPENNYKTTPPVLDSDGSFFLYSRLTVDKSRWQEGNVFSCSVMHEALHNHYTQKSLSLSLGK

SEQ ID NO: 13 - protein, 327 aa, homo sapiens
ASTKGPSVFPLAPCSRSTSESTAALGCLVKDYFPEPVTVSWNSGALTSGVHTFPAVLQSSGLYSLSSVVTVPSSSLGTKTYTCNVDHKPSNTKVDKRVESKYGPPCPPCPAPEFLGGPSVFLFPPKPKDTLMISRTPEVTCVVVDVSQEDPEVQFNWYVDGVEVHNAKTKPREEQFNSTYRVVSVLTVLHQDWLNGKEYKCKVSNKGLPSSIEKTISKAKGQPREPQVYTLPPSQEEMTKNQVSLTCLVKGFYPSDIAVEWESNGQPENNYKTTPPVLDSDGSFFLYSRLTVDKSRWQEGNVFSCSVMHEALHNHYTQKSLSLSPGK

SEQ ID NO: 14 - protein, 327 aa, homo sapiens
ASTKGPSVFPLAPCSRSTSESTAALGCLVKDYFPEPVTVSWNSGALTSGVHTFPAVLQSSGLYSLSSVVTVPSSSLGTKTYTCNVDHKPSNTKVDKRVESKYGPPCPPCPAPEFLGGPSVFLFPPKPKDTLMISRTPEVTCVVVDVSQEDPEVQFNWYVDGVEVHNAKTKPREEQFNSTYRVVSVLTVLHQDWLNGKEYKCKVSNKGLPSSIEKTISKAKGQPREPQVYTLPPSQEEMTKNQVSLTCLVKGFYPSDIAVEWESNGQPENNYKTTPPVLDSDGSFFLYSRLTVDKSRWQEGNVFSCSVMHEALKFHYTQKSLSLSPGK

SEQ ID NO: 15 - protein, 448 aa, artificial
  Artificial
EVQLVQSGAEVKKPGASVKVSCKASGYTFTDYNMDWVRQATGQGLEWIGDINPNYESTGYNQKFKGRATMTVDKSISTAYMELSSLRSEDTAVYYCAREDDHDAFAYWGQGTLVTVSSASTKGPSVFPLAPSSKSTSGGTAALGCLVKDYFPEPVTVSWNSGALTSGVHTFPAVLQSSGLYSLSSVVTVPSSSLGTQTYICNVNHKPSNTKVDKKVEPKSCDKTHTCPPCPAPELLGGPSVFLFPPKPKDTLMISRTPEVTCVVVDVSHEDPEVKFNWYVDGVEVHNAKTKPREEQYNSTYRVVSVLTVLHQDWLNGKEYKCKVSNKALPAPIEKTISKAKGQPREPQVYTLPPSRDELTKNQVSLTCLVKGFYPSDIAVEWESNGQPENNYKTTPPVLDSDGSFFLYSKLTVDKSRWQQGNVFSCSVMHEALHNHYTQKSLSLSPGK

SEQ ID NO: 16 - protein, 447 aa, artificial
  Artificial
EVQLVQSGAEVKKPGASVKVSCKASGYTFTDYNMDWVRQATGQGLEWIGDINPNYESTGYNQKFKGRATMTVDKSISTAYMELSSLRSEDTAVYYCAREDDHDAFAYWGQGTLVTVSSASTKGPSVFPLAPSSKSTSGGTAALGCLVKDYFPEPVTVSWNSGALTSGVHTFPAVLQSSGLYSLSSVVTVPSSSLGTQTYICNVNHKPSNTKVDKKVEPKSCDKTHTCPPCPAPEAAGGPSVFLFPPKPKDTLMISRTPEVTCVVVDVSHEDPEVKFNWYVDGVEVHNAKTKPREEQYNSTYRVVSVLTVLHQDWLNGKEYKCKVSNKALPAPIEKTISKAKGQPREPQVYTLPPSRDELTKNQVSLTCLVKGFYPSDIAVEWESNGQPENNYKTTPPVLDSDGSFFLYSKLTVDKSRWQQGNVFSCSVMHEALKFHYTQKSLSLSPG

SEQ ID NO: 17 - protein, 445 aa, artificial
  Artificial
EVQLVQSGAEVKKPGASVKVSCKASGYTFTDYNMDWVRQATGQGLEWIGDINPNYESTGYNQKFKGRATMTVDKSISTAYMELSSLRSEDTAVYYCAREDDHDAFAYWGQGTLVTVSSASTKGPSVFPLAPCSRSTSESTAALGCLVKDYFPEPVTVSWNSGALTSGVHTFPAVLQSSGLYSLSSVVTVPSSSLGTKTYTCNVDHKPSNTKVDKRVESKYGPPCPSCPAPEFLGGPSVFLFPPKPKDTLMISRTPEVTCVVVDVSQEDPEVQFNWYVDGVEVHNAKTKPREEQFNSTYRVVSVLTVLHQDWLNGKEYKCKVSNKGLPSSIEKTISKAKGQPREPQVYTLPPSQEEMTKNQVSLTCLVKGFYPSDIAVEWESNGQPENNYKTTPPVLDSDGSFFLYSRLTVDKSRWQEGNVFSCSVMHEALHNHYTQKSLSLSLGK

SEQ ID NO: 18 - protein, 445 aa, artificial
  Artificial
EVQLVQSGAEVKKPGASVKVSCKASGYTFTDYNMDWVRQATGQGLEWIGDINPNYESTGYNQKFKGRATMTVDKSISTAYMELSSLRSEDTAVYYCAREDDHDAFAYWGQGTLVTVSSASTKGPSVFPLAPCSRSTSESTAALGCLVKDYFPEPVTVSWNSGALTSGVHTFPAVLQSSGLYSLSSVVTVPSSSLGTKTYTCNVDHKPSNTKVDKRVESKYGPPCPPCPAPEFLGGPSVFLFPPKPKDTLMISRTPEVTCVVVDVSQEDPEVQFNWYVDGVEVHNAKTKPREEQFNSTYRVVSVLTVLHQDWLNGKEYKCKVSNKGLPSSIEKTISKAKGQPREPQVYTLPPSQEEMTKNQVSLTCLVKGFYPSDIAVEWESNGQPENNYKTTPPVLDSDGSFFLYSRLTVDKSRWQEGNVFSCSVMHEALHNHYTQKSLSLSPGK

SEQ ID NO: 19 - protein, 445 aa, artificial
  Artificial
EVQLVQSGAEVKKPGASVKVSCKASGYTFTDYNMDWVRQATGQGLEWIGDINPNYESTGYNQKFKGRATMTVDKSISTAYMELSSLRSEDTAVYYCAREDDHDAFAYWGQGTLVTVSSASTKGPSVFPLAPCSRSTSESTAALGCLVKDYFPEPVTVSWNSGALTSGVHTFPAVLQSSGLYSLSSVVTVPSSSLGTKTYTCNVDHKPSNTKVDKRVESKYGPPCPPCPAPEFLGGPSVFLFPPKPKDTLMISRTPEVTCVVVDVSQEDPEVQFNWYVDGVEVHNAKTKPREEQFNSTYRVVSVLTVLHQDWLNGKEYKCKVSNKGLPSSIEKTISKAKGQPREPQVYTLPPSQEEMTKNQVSLTCLVKGFYPSDIAVEWESNGQPENNYKTTPPVLDSDGSFFLYSRLTVDKSRWQEGNVFSCSVMHEALKFHYTQKSLSLSPGK

SEQ ID NO: 20 - protein, 218 aa, artificial
  Artificial
DNVLTQSPDSLAVSLGERATISCRASKSVRTSGYNYMHWYQQKPGQPPKLLIYLASNLKSGVPDRFSGSGSGTDFTLTISSLQAEDAATYYCQHSRELPYTFGQGTKLEIKRTVAAPSVFIFPPSDEQLKSGTASVVCLLNNFYPREAKVQWKVDNALQSGNSQESVTEQDSKDSTYSLSSTLTLSKADYEKHKVYACEVTHQGLSSPVTKSFNRGEC

SEQ ID NO: 21 - protein, 10 aa, homo sapiens
EPKSCDKTHT

SEQ ID NO: 22 - protein, 5 aa, homo sapiens
CPPCP

SEQ ID NO: 23 - protein, 8 aa, homo sapiens
APELLGGP

SEQ ID NO: 24 - protein, 12 aa, homo sapiens
ELKTPLGDTTHT

SEQ ID NO: 25 - protein, 50 aa, homo sapiens
CPRCPEPKSCDTPPPCPRCPEPKSCDTPPPCPRCPEPKSCDTPPPCPRCP

SEQ ID NO: 26 - protein, 7 aa, homo sapiens
ESKYGPP

SEQ ID NO: 27 - protein, 5 aa, homo sapiens
CPSCP

SEQ ID NO: 28 - protein, 8 aa, homo sapiens
APEFLGGP

SEQ ID NO: 29 - protein, 3 aa, homo sapiens
ERK

SEQ ID NO: 30 - protein, 10 aa, homo sapiens
CCVECPPPCP

SEQ ID NO: 31 - protein, 7 aa, homo sapiens
APPVAGP